European Patent Application EP 4 737 478 A1, published May 6, 2026. Title: 经改造的G蛋白偶联受体及其用途. Applicant: 沃臻生物科技（佛山）有限公司. The sequence listing filed with the application follows.

SEQUENCE LISTING (82 sequences)

SEQ ID NO: 1 - protein, 30 aa, synthetic construct
HYLSTQTSLSKDLNEKRDHMVLLEFVTAAG

SEQ ID NO: 2 - protein, 198 aa, synthetic construct
MGTRKGEELFTGVVPILIELDGDVNGHKFSVRGEGEGDATYGKLTLKFICTTGKLPVPWPTLVTTLTYGVQCFSRYPDHMKRHDFFKSAMPEGYVQERTIYFKDDGTYKTRAEVKFEGDTLVNRIELKGIDFKEDGNILGHKLEYNFNSHNVYIMADKQNNGIKANFKIRHNVEDGSVQLADHYQQNTPIGDGPVLLP

SEQ ID NO: 3 - protein, 332 aa, synthetic construct
PIMGSSVYITVELAIAVLAILGNVLVCWAVWLNSNLQNVTNYFVVSLAAADIAVGVLAIPFAITISTGFCAACHGCLFIACFVLVLTQSSIFSLLAIAIDRYIAIRIPLRYNGLVTGTRAKGIIAICWVLSFAIGLTPMLGWNNCGQPKEGKNHSQGCGEGQVACLFEDVVPMNYMVYFNFFACVLVPLLLMLGVYLRIFLAARRQLGHYLSTQTSLSKDLNEKRDHMVLLEFVTAAGLQKEVHAAKSLAIIVGLFALCWLPLHIINCFTFFCPDCSHAPLWLMYLAIVLSHTNSVVNPFIYAYRIREFRQTFRKIIRSHVLRQQEPFKAAG

SEQ ID NO: 4 - protein, 320 aa, synthetic construct
GRGENFMDIECFMVLNPSQQLAIAVLSLTLGTFTVLENLLVLCVILHSRSLRCRPSYHFIGSLAVADLLGSVIFVYSFIDFHVFHRKDSRNVFLFKLGGVTASFTASVGSLFLAAIDRYISIHRPLAYKRIVTRPKAVVAFCLMWTIAIVIAVLPLLGWNCEKLQSVCSDIFPHIDKTYLMFWIGVVSVLLLFIVYAYMYILWKARRQLGHYLSTQTSLSKDLNEKRDHMVLLEFVTAAGLQKEIELAKTLVLILVVLIICWGPLLAIMVYDVFGKMNKLIKTVFAFCSMLCLLNSTVNPIIYALRSKDLRHAFRSMFPS

SEQ ID NO: 5 - protein, 320 aa, synthetic construct
GRGENFMDIECFMVLNPSQQLAIAVLSLTLGTFTVLENLLVLCVILHSRSLRCRPSYHFIGSLAVADLLGSVIFVYSFIDFHVFHRKDSRNVFLFKLGGVTASFTASVGSLFLAAIDRYISIHRPCAYKRIVTRPKAVVAFCLMWTIAIVIAVLPLLGWNCEKLQSVCSDIFPHIDKTYLMFWIGVVSVLLLFIVYAYMYILWKARRQLGHYLSTQTSLSKDLNEKRDHMVLLEFVTAAGLQKEIELAKTLVLILVVLIICWGPLLAIMVYDVFGKMNKLIKTVFAFCSMLCLLNSTVNPIIYALRSKDLRHAFRSMFPS

SEQ ID NO: 6 - protein, 354 aa, synthetic construct
MDNVLPVDSDLSPNISTNTSEPNQFVQPAWQIVLWAAAYTVIVVTSVVGNVVVMWIILAHKRMRTVTNYFLVNAAFAEASMAAFNTVVNFTYAVHNEWYYGLFYCKFHNFFPIAAIFASIYSMTAVAFDRYMAIIHPCQPRLSLTATKVVICVIWVLALLLAFPQGYYSTTETMPSRVVCKIEWPEHPNKIYEKVYHICVTVLIYFLPLLVIGYLYTVVGITLRRQLGHYLSTQTSLSKDLNEKRDHMVLLEFVTAAGLQKERKVVKMMIVVVCTFAICWLPFHIFLLLPYINPDLYLKKFIQQVYLAIMWLAMSSTMYNPIIYCCLNDRFRLGFKHAFRCCPFISAGDYEGLE

SEQ ID NO: 7 - protein, 332 aa, synthetic construct
PIMGSSVYITVELAIAVLAILGNVLVCWAVWLNSNLQNVTNYFVVSLAAADIAVGVLAIPFAITISTGFCAACHGCLFIACFVLVLTQSSIFSLLAIAIDRYIAIRIPCRYNGLVTGTRAKGIIAICWVLSFAIGLTPMLGWNNCGQPKEGKNHSQGCGEGQVACLFEDVVPMNYMVYFNFFACVLVPLLLMLGVYLRIFLAARRQLGHYLSTQTSLSKDLNEKRDHMVLLEFVTAAGLQKEVHAAKSLAIIVGLFALCWLPLHIINCFTFFCPDCSHAPLWLMYLAIVLSHTNSVVNPFIYAYRIREFRQTFRKIIRSHVLRQQEPFKAAG

SEQ ID NO: 8 - protein, 385 aa, synthetic construct
DYTLDLSVTTVTDYYYPDIFSSPCDAELIQTNGKLLLAVFYCLLFVFSLLGNSLVILVLVVCKKLRSITDVYLLNLALSDLLFVFSFPFQTYYLLDQWVFGTVMCKVVSGFYYIGFYSSMFFITLMSVDRYLAVVHACYALKVRTIRMGTTLCLAVWLTAIMATIPLLVFYQVASEDGVLQCYSFYNQQTLKWKIFTNFKMNILGLLIPFTIFMFCYIKILHQLRRQLGHYLSTQTSLSKDLNEKRDHMVLLEFVTAAGLQKETKAIRLVLIVVIASLLFWVPFNVVLFLTSLHSMHILDGCSISQQLTYATHVTEIISFTHCCVNPVIYAFVGEKFKKHLSEIFQKSCSQIFNYLGRQMPRESCEKSSSCQQHSSRSSSVDYIL

SEQ ID NO: 9 - protein, 379 aa, synthetic construct
YKDCIESTGDYFLLCDAEGPWGIILESLAILGIVVTILLLLAFLFLMRKIQDCSQWNVLPTQLLFLLSVLGLFGLAFAFIIELNQQTAPVRYFLFGVLFALCFSCLLAHASNLVKLVRGCVSFSWTTILCIAIGCSLLQIIIATEYVTLIMTRGMMFVNMTPCQLNVDFVVLLVYVLFLMALTFFVSKATFCGPRRQLGHYLSTQTSLSKDLNEKRDHMVLLEFVTAAGLQKEKQHGRLIFITVLFSIIIWVVWISMLLRGNPQFQRQPQWDDPVVCIALVTNAWVFLLLYIVPELCILYRSCRQECPLQGNACPVTAYQHSFQVENQELSRARDSDGAEEDVALTSYGTPIQPQTVDPTQECFIPQAKLSPQQDAGGV

SEQ ID NO: 10 - protein, 479 aa, synthetic construct
AQVMDFLFEKWKLYGDQCHHNLSLLPPPTELVCNRTFDKYSCWPDTPANTTANISCPWYLPWHHKVQHRFVFKRCGPDGQWVRGPRGQPWRDASQCQMDGEEIEVQKEVAKMYSSFQVMYTVGYSLSLGALLLALAILGGLSKLHCTRNAIHANLFASFVLKASSVLVIDGLLRTRYSQKIGDDLSVSTWLSDGAVAGCRVAAVFMQYGIVANYCWLLVEGLYLHNLLGLACLPERSFFSLYLGIGWGAPMLFVVPWAVVKCLFENVQCWTSNDNMGFWWILRFPVFLAILINFFIFVRIVQLLRRQLGHYLSTQTSLSKDLNEKRDHMVLLEFVTAAGLQKEDYKFRLAKSTLTLIPLLGVHEVVFAFVTDEHAQGTLRSAKLFFDLFLSSFQGLLVAVLYCFLNKEVQSELRRRWHRWRLGKVLWEERNTSNHRASSSPGHGPPSKELQFGRGGGSQDSSAETPLAGGLPRLAESPF

SEQ ID NO: 11 - protein, 424 aa, synthetic construct
SLQDQHCESLSLASNISGLQCNASVDLIGTCWPRSPAGQLVVRPCPAFFYGVRYNTTNNGYRECLANGSWAARVNYSECQEILNEEKKSKVHYHVAVIINYLGHCISLVALLVAFVLFLRLRGGGHYLSTQTSLSKDLNEKRDHMVLLEFVTAAGGGSLRNIIHWNLISAFILRNATWFVVQLTMSPEVHQSNVGWCRLVTAAYNYFHVTNFFWMFGEGCYLHTAIVLTYSTDRLRKWMFICIGWGVPFPIIVAWAIGKLYYDNEKCWFGKRPGVYTDYIYQGPMILVLLINFIFLFNIVRILMTKLRASTTSETIQYRKAVKATLVLLPLLGITYMLFFVNPGEDEVSRVVFIYFNSFLESFQGFFVSVFYCFLNSEVRSAIRKRWHRWQDKHSIRARVARAMSIPTSPTRVSFHSIKQSTAV

SEQ ID NO: 12 - protein, 453 aa, synthetic construct
SLQDQHCESLSLASNISGLQCNASVDLIGTCWPRSPAGQLVVRPCPAFFYGVRYNTTNNGYRECLANGSWAARVNYSECQEILNEEKKSKVHYHVAVIINYLGHCISLVALLVAFVLFLRLRPGCTHWGDQADGALEVGAPWSGAPFQVRRSIRCLRNIIHWNLISAFILRNATWFVVQLTMSPEVHQSNVGWCRLVTAAYNYFHVTNFFWMFGEGCYLHTAIVLTGGGHYLSTQTSLSKDLNEKRDHMVLLEFVTAAGGGDRLRKWMFICIGWGVPFPIIVAWAIGKLYYDNEKCWFGKRPGVYTDYIYQGPMILVLLINFIFLFNIVRILMTKLRASTTSETIQYRKAVKATLVLLPLLGITYMLFFVNPGEDEVSRVVFIYFNSFLESFQGFFVSVFYCFLNSEVRSAIRKRWHRWQDKHSIRARVARAMSIPTSPTRVSFHSIKQSTAV

SEQ ID NO: 13 - protein, 326 aa, synthetic construct
GRAWNRSSYRLHSNASESLGKGYSDGGCYEQLFVSPVVFVTLGVISLLENILVIVAIAKNKNLHSPMYFFICSLAVADMLVSVSLGFETIVITLLNSTDTDAQSFTVNIDNVIDSVICASLLASICSLLSIAVDRYFTIFYALQYHNIMTVKRVGIIISCIWAACTVSGILFIIYSDSSAVIICLITMFFTMLALMASLYVHMFLMARRQLGHYLSTQTSLSKDLNEKRDHMVLLEFVTAAGLQKEMKGAITLTILIGVFVVCWAPFFLHLIFYISCPQNPYCVCFMSHFNLYLILIMCNSIINPLIYALRSQELRKTFKEIICCY

SEQ ID NO: 14 - protein, 347 aa, synthetic construct
MNSTGHLQDAPNATSLHVPHSQEGNSTSLQEGLQDLIHTATLVTCTFLLAVIFCLGSYGNFIVFLSFFDPAFRKFRTNFDFMILNLSFCDLFICGVTAPMFTFVLFFSSASSIPDAFCFTFHLTSSGFIIMSLKTVAVIALHRLRMVLGKQPNRTASFPCTVLLTLLLWATSFTLATLATLKTSKSHLCLPMSSLIAGKGKAILSLYVVDFTFCVAVVSVSYIMIAQTLRKNAGHYLSTQTSLSKDLNEKRDHMVLLEFVTAAGTAKDSKAVVTCVIIVLSVLVCCLPLGISLVQVVLSSNGSFILYQFELFGFTLIFFKSGLNPFIYSRNSAGLRRKVLWCLQYIG

SEQ ID NO: 15 - protein, 334 aa, synthetic construct
GIVNVSERHSCPLGFGHYSVVDVCIFETVVIVLLTFLIIAGNLTVIFVFHCAPLLHHYTTSYFIQTMAYADLFVGVSCLVPTLSLLHYSTGVHESLTCQVFGYIISVLKSVSMWCLACISVDRYLAITKPCSYNQLVTPCRLRICIILIWIYSCLIFLPSFFGWGKPGYHGDIFEWCATSWLTSAYFTGFIVCLLYAPAAFVVCFTYFHIFKICRRQLGHYLSTQTSLSKDLNEKRDHMVLLEFVTAAGLQKERRYLMVLFRITSVFYMLWLPYIIYFLLESSRVLDNPTLSFLTTWLAISNSFCNPVIYALSDSTFRLGLRRLSETMCTSCMC

SEQ ID NO: 16 - protein, 344 aa, synthetic construct
MANSASPEQNQNHCSAINNSIPLMQGNLPTLTLSGKIRVTVTFFLFLLSATFNASFLLKLQKWTQKKEKGKKLSRMKLLLKHLTLANLLETLIVMPLDGMWNITVQWYAGELLCKVLSYLKLFSMYAKAFMMVVISLDRSLAITRPCALKSNSKVGQSMVGLAWILSSVFAGPQLYIFRMIHLADSSGQTKVFSQCVTHCSFSQWWHQAFYNFFTFSCLFIIPLFIMLICNAKIIFTLRRQLGHYLSTQTSLSKDLNEKRDHMVLLEFVTAAGLQKERLKTLKMTVAFATSFTVCWTPYYVLGIWYWFDPEMLNRLSDPVNHFFFLFAFLNPCFDPLIYGYFSL

SEQ ID NO: 17 - protein, 370 aa, synthetic construct
MSANATLKPLCPILEQMSRLQSHSNTSIRYIDHAAVLLHGLASLLGLVENGVILFVVGCRMRQTVVTTWVLHLALSDLLASASLPFFTYFLAVGHSWELGTTFCKLHSSIFFLNMFASGFLLSAISLDRCLQVVRPCWAQNHRTVAAAHKVCLVLWALAVLNTVPYFVFRDTISRLDGRIMCYYNVLLLNPGPDRDATCNSRQVALAVSKFLLAFLVPLAIIASSHAAVSLRLQHRGGHYLSTQTSLSKDLNEKRDHMVLLEFVTAAGRRRPGRFVRLVAAVVAAFALCWGPYHVFSLLEARAHANPGLRPLVWRGLPFVTSLAFFNSVANPVLYVLTCPDMLRKLRRSLRTVLESVLVDDSELGGAGSS

SEQ ID NO: 18 - protein, 331 aa, synthetic construct
GAPTSDGGRFKFPDGVQNWPALSIVIIIIMTIGGNILVIMAVSMEKKLHNATNYFLMSLAIADMLVGLLVMPLSLLAILYDYVWPLPRYLCPVWISLDVLFSTASIMHLCAISLDRYVAIRNPCEHSRFNSRTKAIMKIAIVWAISIGVSVPIPVIGLRDEEKVFVNNTTCVLNDPNFVLIGSFVAFFIPLTIMVITYCLTIYVLRRQLGHYLSTQTSLSKDLNEKRDHMVLLEFVTAAGLQKERKASKVLGIVFFVFLIMWCPFFITNILSVLCEKSCNQKLMEKLLNVFVWIGYVNSGINPLVYTLFNKIYRRAFSNYLRCNYKVEKKP

SEQ ID NO: 19 - protein, 315 aa, synthetic construct
SVQATAAIAAAITFLILFTIFGNALVILAVLTSRSLRAPQNLFLVSLAAADILVATLIIPFSLANELLGYWYFRRTWCEVYLALDVLFCTSSIVHLCAISLDRYWAVSRACEYNSKRTPRRIKCIILTVWLIAAVISLPPLIYKGDQGPQPRGRPQCKLNQEAWYILASSIGSFFAPCLIMILVYLRIYLIARRQLGHYLSTQTSLSKDLNEKRDHMVLLEFVTAAGLQKEKRFTFVLAVVIGVFVLCWFPFFFSYSLGAICPKHCKVPHGLFQFFFWIGYCNSSLNPVIYTIFNQDFRRAFRRILCRPWTQTAW

SEQ ID NO: 20 - protein, 325 aa, synthetic construct
ASESPEPLSQQWTAGMGLLMALIVLLIVAGNVLVIVAIAKTPRLQTLTNLFIMSLASADLVMGLLVVPFGATIVVWGRWEYGSFFCELWTSVDVLCVTASIETLCVIALDRYLAITSPCRYQSLLTRARARGLVCTVWAISALVSFLPILMHWWRAESDEARRCYNDPKCCDFVTNRAYAIASSVVSFYVPLCIMAFVYLRVFREARRQLGHYLSTQTSLSKDLNEKRDHMVLLEFVTAAGLQKEQKALKTLGIIMGVFTLCWLPFFLANVVKAFHRELVPDRLFVFFNWLGYANSAFNPIIYCRSPDFRKAFQGLLCCARRAAR

SEQ ID NO: 21 - protein, 336 aa, synthetic construct
AADEVWVVGMGIVMSLIVLAIVFGNVLVITAIAKFERLQTVTNYFITSLACADLVMGLAVVPFGAAHILTKTWTFGNFWCEFWTSIDVLCVTASIETLCVIAVDRYFAITSPCKYQSLLTKNKARVIILMVWIVSGLTSFLPIQMHWYRATHQEAINCYAEETCCDFFTNQAYAIASSIVSFYVPLVIMVFVYSRVFQEARRQLGHYLSTQTSLSKDLNEKRDHMVLLEFVTAAGLQKEHKALKTLGIIMGTFTLCWLPFFIVNIVHVIQDNLIRKEVYILLNWIGYVNSGFNPLIYCRSPDFRIAFQELLCLRRSSLKAYGNGYSSNGNTGEQSG

SEQ ID NO: 22 - protein, 332 aa, synthetic construct
SNTLRVPDILALVIFAVVFLVGVLGNALVVWVTAFEAKRTINAIWFLNLAVADFLSCLALPILFTSIVQHHHWPFGGAACSILPSLILLNMYASILLLATISADRFLLVFKPCWCQNFRGAGLAWIACAVAWGLALLLTIPSFLYRVVREEYFPPKVLCGVDYSHDKRRERAVAIVRLVLGFLWPLLTLTICYTFILLRTRRQLGHYLSTQTSLSKDLNEKRDHMVLLEFVTAAGLQKETKTLKVVVAVVASFFIFWLPYQVTGIMMSFLEPSSPTFLLLKKLDSLCVSFAYINCCINPIIYVVAGQGFQGRLRKSLPSLLRNVLTEESVVR

SEQ ID NO: 23 - protein, 361 aa, synthetic construct
GTLSTSRSRFIRNTNESGEEVTTFFDYDYGAPCHKFDVKQIGAQLLPPLYSLVFIFGFVGNMLVVLILINCKKLKCLTDIYLLNLAISDLLFLITLPLWAHSAANEWVFGNAMCKLFTGLYHIGYFGGIFFIILLTIDRYLAIVHACFALKARTVTFGVVTSVITWLVAVFASVPGIIFTKCQKEDSVYVCGPYFPRGWNNFHTIMRNILGLVLPLLIMVICYSGISRASRRQLGHYLSTQTSLSKDLNEKRDHMVLLEFVTAAGLQKEKKAVRVIFTIMIVYFLFWTPYNIVILLNTFQEFFGLSNCESTSQLDQATQVTETLGMTHCCINPIIYAFVGEKFRRYLSVFFRKHITKRFGR

SEQ ID NO: 24 - protein, 393 aa, synthetic construct
GAPDYQVSSPIYDINYYTSEPCQKINVKQIAARLLPPLYSLVFIFGFVGNMLVILILINYKRLKSMTDIYLLNLAISDLFFLLTVPFWAHYAAAQWDFGNTMCQLLTGLYFIGFFSGIFFIILLTIDRYLAVVHACFALKARTVTFGVVTSVITWVVAVFASLPNIIFTRSQKEGLHYTCSSHFPYSQYQFWKNFQTLKIVILGLVLPLLVMVICYSGILKTLRRQLGHYLSTQTSLSKDLNEKRDHMVLLEFVTAAGLQKEHRDVRLIFTIMIVYFLFWAPYNIVLLLNTFQEFFGLNNCSSSNRLDQAMQVTETLGMTHCCINPIIYAFVGEEFRNYLLVFFQKHIAKRFCKCCSIFQQEAPERASSVYTRSTGEQEISVGLGRPLEVLFQ

SEQ ID NO: 25 - protein, 404 aa, synthetic construct
SGESMNFSDVFDSSEDYFVSVNTSYYSVDSEMLLCSLQEVRQFSRLFVPIAYSLICVFGLLGNILVVITFAFYKKARSMTDVYLLNMAIADILFVLTLPFWAVSHATGAWVFSNATCKLLKGIYAINFNCGMLLLTCISMDRYIAIVQACKSFRLRSRTLPRSKIICLVVWGLSVIISSSTFVFNQKYNTQGSDVCEPKYQTVSEPIRWKLLMLGLELLFGFFIPLMFMIFCYTFIVKTLRRQLGHYLSTQTSLSKDLNEKRDHMVLLEFVTAAGLQKEHKAIRVIIAVVLVFLACQIPHNMVLLVTAANLGKMNRSCQSEKLIGYTKTVTEVLAFLHCCLNPVLYAFIGQKFRNYFLKILKDLWCVRRKYKSSGFSCAGRYSENISRQTSETADNDNASSFTM

SEQ ID NO: 26 - protein, 347 aa, synthetic construct
GPGSSLCSKKDVRNFKAWFLPIMYSIICFVGLLGNGLVVLTYIYFKRLKTMTDTYLLNLAVADILFLLTLPFWAYSAAKSWVFGVHFCKLIFAIYKMSFFSGMWLLLCISIDRYVAIVQACSAHRHRARVLLISKLSCVGIWILATVLSIPELLYSDLQRSSSEQAMRCSLITEHVEAFITIQVAQMVIGFLVPLLAMSFCYLVIISKLRRQLGHYLSTQTSLSKDLNEKRDHMVLLEFVTAAGLQKENKAIKVIIAVVVVFIVFQLPYNGVVLAQTVANFNITSSTCELSKQLNIAYDVTYSLACVRCCVNPFLYAFIGVKFRNDLFKLFKDLGCLSGGRLEVLFQ

SEQ ID NO: 27 - protein, 338 aa, synthetic construct
GPMDDSTDSSDNSLALTSPYKTFEVVFIVLVAGSLSLVTIIGNILVMVSIKVNRHLQTVNNYFLFSLACADLIIGVFSMNLYTLYTVIGYWPLGPVVCDLWLALDYVVSNARVMNLLIISFDRYFCVTKPCTYPVKRTTKMAGMMIAAAWVLSFILWAPAILFWQFIVGVRTVEDGECYIQFFSNAAVTFGTAIAAFYLPVIIMTVLYWHISRASRRQLGHYLSTQTSLSKDLNEKRDHMVLLEFVTAAGLQKEKKVTRTILAILLAFIITWAPYNVMVLINTFCAPCIPNTVWTIGYWLCYINSTINPACYALCNATFKKTFKHLLMCHYKNIGATR

SEQ ID NO: 28 - protein, 331 aa, synthetic construct
MEPNGTFSNNNSRNCTIENFKREFFPIVYLIIFFVGVLGNGLSIYVFLQPYKKSTSVNVFMLNLAISNLLFISTLPFRADYYLRGSNWIFGDLACRIMSYSLYVNMYSSIYFLTVLSVVRYLAMVHPCRLLHVTSIRSAWILCGIIWILIMASSIMLLDSGSEQNGSVTSCLELNLYKIAKLQTMNYIALVVGCLLPFFTLSICYLLIIRVLRRQLGHYLSTQTSLSKDLNEKRDHMVLLEFVTAAGLQKERKALTTIIITLIIFFLCFLPYHTLRTVHLTTWKVGLCKDRLHKALVITLALAAANACFNPLLYYFAGENFKDRLKSALRK

SEQ ID NO: 29 - protein, 339 aa, synthetic construct
APCEPESLEINKYFVVIIYALVFLLSLLGNSLVMLVILYSRVGRSVTDVYLLNLALADLLFALTLPIWAASKVNGWIFGTFLCKVVSLLKEVNFYSGIWLLACISVDRYLAIVHACRTLTQKRYLVKFICLSIWGLSLLLALPVLLFRRTVYSSNVSPACYEDMGNNTANWRMLLRILPQSFGFIVPLLIMLFCYGFTLRTLRRQLGHYLSTQTSLSKDLNEKRDHMVLLEFVTAAGLQKEHREMRVIFAVVLIFLLCWLPYNLVLLADTLMRTQVIQETCERRNHIDRALDATEILAILHSCLNPLIYAFIGQKFRHGLLKILAIHGLISKDSLPKDS

SEQ ID NO: 30 - protein, 359 aa, synthetic construct
AGAPEGISIYTSDNYTEEMGSGDYDSMKEPCFREENANFNKIFLPTIYSIIFLTGIVGNGLVILVMGYQKKLRSMTDKYRLHLSVADLLFVITLPFWAVDAVANWYFGNFLCKAVHVIYTVNLYSSVWILAFISLDRYLAIVHACNSQRPRKLLAEKVVYVGVWIPALLLTIPDFIFANVSEADDRYICDRFYPNDLWVVVFQFQHIMVGLILPGIVILSCYCIIISKLRRQLGHYLSTQTSLSKDLNEKRDHMVLLEFVTAAGLQKERKALKTTVILILAFFACWLPYYIGISIDSFILLEIIKQGCEFENTVHKWISITEALAFFHCCLNPILYAFLGAKFKTSAQHALTSVSRGSS

SEQ ID NO: 31 - protein, 297 aa, synthetic construct
YNYYATLLTLLIAVIVFGNVLVCMAVSREKALQTTTNYLIVSLAVADLLVATLVMPWVVYLEVVGEWKFSRIHCDIFVTLDVMMCTASALNLCAISIDRYTAVAMPCLYNTRYSSKRRVTVMISIVWVLSFTISCPLLFGLNNADQNECIIANPAFVVYSSIVSFYVPFIVTLLVYIKIYIVLRRQLGHYLSTQTSLSKDLNEKRDHMVLLEFVTAAGLQKEKKATQMAAIVAGVFIICWLPFFITHILNIHCDCNIPPVLYSAFTWLGYVNSAVNPIIYTTFNIEFRKAFLKILHC

SEQ ID NO: 32 - protein, 331 aa, synthetic construct
APASLSQLSSHLNYTCGAENSTGASQARPHAYYALSYCALILAIVFGNGLVCMAVLKERALQTTTNYLVVSLAVADLLVATLVMPWVVYLEVTGGVWNFSRICCDVFVTLDVMMCTASIWNLCAISIDRYTAVVMPCHYQHGTGQSSCRRVALMITAVWVLAFAVSCPLLFGFNTTGDPTVCSISNPDFVIYSSVVSFYLPFGVTVLVYARIYVVLRRQLGHYLSTQTSLSKDLNEKRDHMVLLEFVTAAGLQKEKKATQMVAIVLGAFIVCWLPFFLTHVLNTHCQTCHVSPELYSATTWLGYVNSALNPVIYTTFNIEFRKAFLKILSC

SEQ ID NO: 33 - protein, 342 aa, synthetic construct
MTPNSTGEVPSPIPKGALGLSLALASLIITANLLLALGIAWDRRLRSPPAGCFFLSLLLAGLLTGLALPTLPGLWNQSRRGYWSCLLVYLAPNFSFLSLLANLLLVHGERYMAVLRPCQPPGSIRLALLLTWAGPLLFASLPALGWNHWTPGANCSSQAIFPAPYLYLEVYGLLLPAVGAAAFLSVRVLATARRQLGHYLSTQTSLSKDLNEKRDHMVLLEFVTAAGLQKEWRQARAQAGAMLLFGLCWGPYVATLLLSVLAYEQRPPLGPGTLLSLLSLGSASAAAVPVAMGLGDQRYTAPWRAAAQRCLQGLWGRASRDSPGPSIAYHPSSQSSVDLDLN

SEQ ID NO: 34 - protein, 314 aa, synthetic construct
TTMASPQLMPLVVVLSTICLVTVGLNLLVLYAVRSERKLHTVGNLYIVSLSVADLIVGAVVMPMNILYLLMSKWSLGRPLCLFWLSMDYVASTASIFSVFILCIDRYRSVQQPCRYLKYRTKTRASATILGAWFLSFLWVIPILGWNHFMQQTSVRREDKCETDFYDVTWFKVMTAIINFYLPTLLMLWFYAKIYKAVRRQLGHYLSTQTSLSKDLNEKRDHMVLLEFVTAAGLQKERKAAKQLGFIMAAFILCWIPYFIFFMVIAFCKNCCNEHLHMFTIWLGYINSTLNPLIYPLCNENFKKTFKRILHIRS

SEQ ID NO: 35 - protein, 321 aa, synthetic construct
GTTTGISDVTVSYQVITSLLLGTLIFCAVLGNACVVAAIALERSLQNVANYLIGSLAVTDLMVSVLVLPMAALYQVLNKWTLGQVTCDLFIALDVLCCTSSIWHLCAIALDRYWAITDPCDYVNKRTPRRAAALISLTWLIGFLISIPPMLGWRTPEDRSDPDACTISKDHGYTIYSTFGAFYIPLLLMLVLYGRIFRAARRQLGHYLSTQTSLSKDLNEKRDHMVLLEFVTAAGLQKERKTVKTLGIIMGTFILCWLPFFIVALVLPFCESSCHMPTLLGAIINWLGYSNSLLNPVIYAYFNKDFQNAFKKIIKCKFCRQ

SEQ ID NO: 36 - protein, 325 aa, synthetic construct
GTCSAKDYIYQDSISLPWKVLLVMLLALITLATTLSNAFVIATVYRTRKLHTPANYLIASLAVTDLLVSILVMPISTMYTVTGRWTLGQVVCDFWLSSDITCCTASIWHLCVIALDRYWAITDACEYSAKRTPKRAAVMIALVWVFSISISLPPFFWRQAKAEEEVSECVVNTDHILYTVYSTVGAFYFPTLLLIALYGRIYVEARRQLGHYLSTQTSLSKDLNEKRDHMVLLEFVTAAGLQKERKATKTLGIILGAFIVCWLPFFIISLVMPICKDACWFHLAIFDFFTWLGYLNSLINPIIYTMSNEDFKQAFHKLIRFKCTS

SEQ ID NO: 37 - protein, 337 aa, synthetic construct
GAPTESIPEEMKQIVEEQGNKLHWAALLILMVIIPTIGGNTLVILAVSLEKKLQYATNYFLMSLAVADLLVGLFVMPIALLTIMFEAMWPLPLVLCPAWLFLDVLFSTASIWHLCAISVDRYIAIKKPCQANQYNSRATAFIKITVVWLISIGIAIPVPIKGIETDVDNPNNITCVLTKERFGDFMLFGSLAAFFTPLAIMIVTYFLTIHALRRQLGHYLSTQTSLSKDLNEKRDHMVLLEFVTAAGLQKEQRASKVLGIVFFLFLLMWCPFFITNITLVLCDSCNQTTLQMLLEIFVWIGYVSSGVNPLVYTLFNKTFRDAFGRYITCNYRATKSV

SEQ ID NO: 38 - protein, 342 aa, synthetic construct
STSIPVISQPQFTAMNEPQCFYNESIAFFYNRSGKHLATEWNTVSKLVMGLGITVCIFIMLANLLVMVAIYVNRRFHFPIYYLMANLAAADFFAGLAYFYLMFNTGPNTRRLTVSTWLLRQGLIDTSLTASVANLLAIAIERHITVFRMCLHTRMSNRRVVVVIVVIWTMAIVMGAIPSVGWNCICDIENCSNMAPLYSDSYLVFWAIFNLVTFVVMVVLYAHIFGYVRRQLGHYLSTQTSLSKDLNEKRDHMVLLEFVTAAGLQKEMSLLKTVVIVLGAFIICWTPGLVLLLLDVCCPQCDVLAYEKFFLLLAEFNSAMNPIIYSYRDKEMSATFRQILGR

SEQ ID NO: 39 - protein, 330 aa, synthetic construct
GDGARPSWVAPALSAVLIVTTAVDVVGNLLVILSVLRNRKLRNAGNLFLVSLALANLVVAFYPYPLILVAIFYDGWAFGEEHCKASAFVMGLSVIGSVWNITAIAIDRYLYICHSCAYHRIYRRWHTPLHICLIWLLTVVALLPNFFVGSLEYDPRIYSCTFIQTASTQYTAAVVVIAFLLPIAVVSFCYLRIWVLVRRQLGHYLSTQTSLSKDLNEKRDHMVLLEFVTAAGLQKELRSFLTMFVVFVIFAICFAPLNCIGLAVAINPQEMAPQIPEGLFVTSYLLAYFNSCLNPIVYGLLDQNFRREYKRILLALWNPRHCIQDASKGS

SEQ ID NO: 40 - protein, 378 aa, synthetic construct
APNSTLFSQVENHSVHSNFSEKNAQLLAFENDDCHLPLAMIFTLALAYGAVIILGVSGNLALIIIILKQKEMRNVTNILIVNLSFSDLLVAIMCLPFTFVYTLMDHWVFGEAMCKLNPFVQCVSITVSIWSLVLIAVERHQLIINPCGWRPNNRHAYVGIAVIWVLAVASSLPFLIYQVMTDEPFQNVTLDAYKDKYVCFDQFPSDSHRLSYTTLLLVLQYFGPLCFIFICYFKIYIRLRRQLGHYLSTQTSLSKDLNEKRDHMVLLEFVTAAGLQKEKRINIMLLSIVVAFAVCWLPLTIFNTVFDWNHQIIATCNHNLLFLLCHLTAMISTCVNPIFYGFLNKNFQRDLQFFFNFCDFRSRDDDYETIAMSTMHTD

SEQ ID NO: 41 - protein, 324 aa, synthetic construct
PGARSASSLALAIAITALYSAVCAVGLLGNVLVMFGIVRYTKMKTATNIYIFNLALADALATSTLPFQSAKYLMETWPFGELLCKAVLSIDYYNMFTSIFTLTMMSVDRYIAVCHPCKALDFRTPAKAKLINICIWVLASGVGVPIMVMAVTRPRDGAVVCMLQFPSPSWYWDTVTKICVFLFAFVVPILIITVCYGLMLLRLRRQLGHYLSTQTSLSKDLNEKRDHMVLLEFVTAAGLQKERRITRMVLVVVGAFVVCWAPIHIFVIVWTLVDIDRRDPLVVAALHLCIALGYANSSLNPVLYAFLDENFKRCFRQLCRKPCG

SEQ ID NO: 42 - protein, 375 aa, synthetic construct
MGTKLEDSPPCRNWSSASELNETQEPFLNPTDYDDEEFLRYLWREYLHPKEYEWVLIAGYIIVFVVALIGNVLVCVAVWKNHHMRTVTNYFIVNLSLADVLVTITCLPATLVVDITETWFFGQSLCKVIPYLQTVSVSVSVLTLSCIALDRWYAICHPCMFKSTAKRARNSIVIIWIVSCIIMIPQAIVMECSTVFPGLANKTTLFTVCDERWGGEIYPKMYHICFFLVTYMAPLCLMVLAYLQIFRKLRRQLGHYLSTQTSLSKDLNEKRDHMVLLEFVTAAGLQKERKTARMLMVVLLVFAICYLPISILNVLKRVFGMFAHTEDRETVYAWFTFSHWLVYANSAANPIIYNFLSGKFREEFKAAFSCCCLGV

SEQ ID NO: 43 - protein, 367 aa, synthetic construct
MKSPFYRCQNTTSVEKGNSAVMGGVLFSTGLLGNLLALGLLARSGLGWCSRRPLRPLPSVFYMLVCGLTVTDLLGKCLLSPVVLAAYAQNRSLRVLAPALDNSLCQAFAFFMSFFGLSSTLQLLAMALECWLSLGHPCFYRRHITLRLGALVAPVVSAFSLAFCALPFMGFGKFVQYCPGTWCFIQMVHEEGSLSVLGYSVLYSSLMALLVLATVLCNLGAMRNLYAMHRRLQGHYLSTQTSLSKDLNEKRDHMVLLEFVTAAGPLEELDHLLLLALMTVLFTMCSLPVIYRAYYGAFKDVKEKNRTSEEAEDLRALRFLSVISIVDPWIFIIFRSPVFRIFFHKIFIRPLRYRSRCSNSTNMESSL

SEQ ID NO: 44 - protein, 358 aa, synthetic construct
MWSCSWFNGTGLVEELPACQDLQLGLSLLSLLGLVVGVPVGLCYNALLVLANLHSKASMTMPDVYFVNMAVAGLVLSALAPVHLLGPPSSRWALWSVGGEVHVALQIPFNVSSLVAMYSTALLSLDHYIERALPCTYMASVYNTRHVCGFVWGGALLTSFSSLLFYICSHVSTRALECAKMQNAEAADATLVFIGYVVPALATLYALVLLSRVRRRQLGHYLSTQTSLSKDLNEKRDHMVLLEFVTAAGLQKEPSAHRLLVATVCTQFGLWTPHYLILLGHTVIISRGKPVDAHYLGLLHFVKDFSKLLAFSSSFVTPLLYRYMNQSFPSKLQRLMKKLPCGDRHCSPDHMGVQQVLA

SEQ ID NO: 45 - protein, 376 aa, synthetic construct
MDLEASLLPTGPNASNTSDGPDNLTSAGSPPRTGSISYINIIMPSVFGTICLLGIIGNSTVIFAVVKKSKLHWCNNVPDIFIINLSVVDLLFLLGMPFMIHQLMGNGVWHFGETMCTLITAMDANSQFTSTYILTAMAIDRYLATVHPCSSTKFRKPSVATLVICLLWALSFISITPVWLYARLIPFPGGAVGCGIRLPNPDTDLYWFTLYQFFLAFALPFVVITAAYVRILQRMTSSVGHYLSTQTSLSKDLNEKRDHMVLLEFVTAAGRLRTKRVTRTAIAICLVFFVCWAPYYVLQLTQLSISRPTLTFVYLYNAAISLGYANSCLNPFVYIVLCETFRKRLVLSVKPAAQGQLRAVSNAQTADEERTESKGT

SEQ ID NO: 46 - protein, 350 aa, synthetic construct
MMPFCHNIINISCVKNNWSNDVRASLYSLMVLIILTTLVGNLIVIVSISHFKQLHTPTNWLIHSMATVDFLLGCLVMPYSMVRSAEHCWYFGEVFCKIHTSTDIMLSSASIFHLSFISIDRYYAVCDPCRYKAKMNILVICVMIFISWSVPAVFAFGMIFLELNFKGAEEIYYKHVHCRGGCSVFFSKISGVLTFMTSFYIPGSIMLCVYYRIYLIAKEQARGHYLSTQTSLSKDLNEKRDHMVLLEFVTAAGQSKERKAVKTLGIVMGVFLICWCPFFICTVMDPFLHYIIPPTLNDVLIWFGYLNSTFNPMVYAFFYPWFRKALKMMLFGKIFQKDSSRCKLFLELSS

SEQ ID NO: 47 - protein, 385 aa, synthetic construct
MILNSSTEDGIKRIQDDCPKAGRHNYIFVMIPTLYSIIFVVGIFGNSLVVIVIYFYMKLKTVASVFLLNLALADLCFLLTLPLWAVYTAMEYRWPFGNYLCKIASASVSFNLYASVFLLTCLSIDRYLAIVHPCKSRLRRTMLVAKVTCIIIWLLAGLASLPAIIHRNVFFIENTNITVCAFHYESQNSTLPIGLGLTKNILGFLFPFLIILTSYTLIWKALKKAYGHYLSTQTSLSKDLNEKRDHMVLLEFVTAAGKPRNDDIFKIIMAIVLFFFFSWIPHQIFTFLDVLIQLGIIRDCRIADIVDTAMPITICIAYFNNCLNPLFYGFLGKKFKRYFLQLLKYIPPKAKSHSNLSTKMSTLSYRPSDNVSSSTKKPAPCFEVE

SEQ ID NO: 48 - protein, 381 aa, synthetic construct
METNSSLPTNISGGTPAVSAGYLFLDIITYLVFAVTFVLGVLGNGLVIWVAGFRMTHTVTTISYLNLAVADFCFTSTLPFFMVRKAMGGHWPFGWFLCKFVFTIVDINLFGSVFLIALIALDRCVCVLHPCWTQNHRTVSLAKKVIIGPWVMALLLTLPVIIRVTTVPGKTGTVACTFNFSPWTNDPKERINVAVAMLTVRGIIRFIIGFSAPMSIVAVSYGLIATKIHKQGGHYLSTQTSLSKDLNEKRDHMVLLEFVTAAGLIKSSRPLRVLSFVAAAFFLCWSPYQVVALIATVRIRELLQGMYKEIGIAVDVTSALAFFNSCLNPMLYVFMGQDFRERLIHALPASLERALTEDSTQTSDTATNSTLPSAEVELQAK

SEQ ID NO: 49 - protein, 373 aa, synthetic construct
MELAVGNLSEGNASWPEPPAPEPGPLFGIGVENFVTLVVFGLIFALGVLGNSLVITVLARSKPGKPRSTTNLFILNLSIADLAYLLFCIPFQATVYALPTWVLGAFICKFIHYFFTVSMLVSIFTLAAMSVDRYVAIVHSCRSSSLRVSRNALLGVGCIWALSIAMASPVAYHQGLFHPRASNQTFCWEQWPDPRHKKAYVVCTFVFGYLLPLLLICFCYAKVLNHLHKKLGHYLSTQTSLSKDLNEKRDHMVLLEFVTAAGEASKKKTAQTVLVVVVVFGISWLPHHIIHLWAEFGVFPLTPASFLFRITAHCLAYSNSSVNPIIYAFLSENFRKAYKQVFKCHIRKDSHLSDTKESKSRIDTPPSTNCTHV

SEQ ID NO: 50 - protein, 386 aa, synthetic construct
MWNATPSEEPGFNLTLADLDWDASPGNDSLGDELLQLFPAPLLAGVTATCVALFVVGIAGNLLTMLVVSRFRELRTTTNLYLSSMAFSDLLIFLCMPLDLVRLWQYRPWNFGDLLCKLFQFVSESCTYATVLTITALSVERYFAICFPCRAKVVVTKGRVKLVIFVIWAVAFCSAGPIFVLVGVEHENGTDPWDTNECRPTEFAVRSGLLTVMVWVSSIFFFLPVFCLTVLYSLIGRKLRRQLGHYLSTQTSLSKDLNEKRDHMVLLEFVTAAGLQKEKQTVKMLAVVVFAFILCWLPFHVGRYLFSKSFEPGSLEIAQISQYCNLVSFVLFYLSAAINPILYNIMSKKYRVAVFRLLGFEPFSQRKLSTLKDESSRAWTESSINT

SEQ ID NO: 51 - protein, 395 aa, synthetic construct
MDVVDSLLVNGSNITPPCELGLENETLFCLDQPRPSKEWQPAVQILLYSLIFLLSVLGNTLVITVLIRNKRMRTVTNIFLLSLAVSDLMLCLFCMPFNLIPNLLKDFIFGSAVCKTTTYFMGTSVSVSTFNLVAISLERYGAICKPCQSRVWQTKSHALKVIAATWCLSFTIMTPYPIYSNLVPFTKNNNQTANMCRFLLPNDVMQQSWHTFLLLILFLIPGIVMMVAYGLISLELYQGIGHYLSTQTSLSKDLNEKRDHMVLLEFVTAAGLMAKKRVIRMLIVIVVLFFLCWMPIFSANAWRAYDTASAERRLSGTPISFILLLSYTSSCVNPIIYCFMNKRFRLGFMATFPCCPNPGPPGARGEVGEEEEGGTTGASLSRFSYSHMSASVPPQ

SEQ ID NO: 52 - protein, 432 aa, synthetic construct
MGSPWNGSDGPEGAREPPWPALPPCDERRCSPFPLGALVPVTAVCLCLFVVGVSGNVVTVMLIGRYRDMRTTTNLYLGSMAVSDLLILLGLPFDLYRLWRSRPWVFGPLLCRLSLYVGEGCTYATLLHMTALSVERYLAICRPCRARVLVTRRRVRALIAVLWAVALLSAGPFLFLVGVEQDPGISVVPGLNGTARIASSPLASSPPLWLSRAPPPSPPSGPETAEAAALFSRECRPSPAQLGALRVMLWVTTAYFFLPFLCLSILYGLIGRELRRQLGHYLSTQTSLSKDLNEKRDHMVLLEFVTAAGLQKERQTVRVLLVVVLAFIICWLPFHVGRIIYINTEDSRMMYFSQYFNIVALQLFYLSASINPILYNLISKKYRAAAFKLLLARKSRPRGFHRSRDTAGEVAGDTGGDTVGYTETSANVKTMG

SEQ ID NO: 53 - protein, 427 aa, synthetic construct
DNPERYSTNLSNHVDDFTTFRGTELSFLVTTHQPTNLVLPSNGSMHNYCPQQTKITSAFKYINTVISCTIFIVGMVGNATLLRIIYQNKCMRNGPNALIASLALGDLIYVVIDLPINVFKLLAGRWPFDHNDFGVFLCKLFPFLQKSSVGITVLNLCALSVDRYRAVASWCRVQGIGIPLVTAIEIVSIWILSFILAIPEAIGFVMVPFEYRGEQHKTCMLNATSKFMEFYQDVKDWWLFGFYFCMPLVCTAIFYTLMTCEMLNRRGHYLSTQTSLSKDLNEKRDHMVLLEFVTAAGLKQRREVAKTVFCLVVIFALCWFPLHLSRILKKTVYNEMDKNRCELLSFLLLMDYIGINLATMNSCINPIALYFVSKKFKNCFQSCLCCCCYQSKSLMTSVPMNGTSIQWKNHDQNNHNTDRSSHKDSMN

SEQ ID NO: 54 - protein, 390 aa, synthetic construct
MASSTTRGPRVSDLFSGLPPAVTTPANQSAEASAGNGSVAGADAPAVTPFQSLQLVHQLKGLIVLLYSVVVVVGLVGNCLLVLVIARVRRLHNVTNFLIGNLALSDVLMCTACVPLTLAYAFEPRGWVFGGGLCHLVFFLQPVTVYVSVFTLTTIAVDRYVVLVHPCRRRISLRLSAYAVLAIWALSAVLALPAAVHTYHVELKPHDVRLCEEFWGSQERQRQLYAWGLLLVTYLLPLLVILLSYVRVSVKLRNRVGHYLSTQTSLSKDLNEKRDHMVLLEFVTAAGGGRARRRRTFCLLVVIVVVFAVCWLPLHVFNLLRDLDPHAIDPYAFGLVQLLCHWLAMSSACYNPFIYAWLHDSFREELRKLLVAWPRKIAPHGQNMTVSVVI

SEQ ID NO: 55 - protein, 377 aa, synthetic construct
MEGEPSQPPNSSWPLSQNGTNTEATPATNLTFSSYYQHTSPVAAMFIVAYALIFLLCMVGNTLVCFIVLKNRHMHTVTNMFILNLAVSDLLVGIFCMPTTLVDNLITGWPFDNATCKMSGLVQGMSVSASVFTLVAIAVERFRCIVHPCREKLTLRKALVTIAVIWALALLIMCPSAVTLTVTREEHHFMVDARNRSYPLYSCWEAWPEKGMRRVYTTVLFSHIYLAPLALIVVMYARIARKLCQAPGHYLSTQTSLSKDLNEKRDHMVLLEFVTAAGGGSRRRARVVHMLVMVALFFTLSWLPLWALLLLIDYGQLSAPQLHLVTVYAFPFAHWLAFFNSSANPIIYGYFNENFRRGFQAAFRARLCPRPSGSHKE

SEQ ID NO: 56 - protein, 383 aa, synthetic construct
MSNITDPQMWDFDDLNFTGMPPADEDYSPCMLETETLNKYVVIIAYALVFLLSLLGNSLVMLVILYSRVGRSVTDVYLLNLALADLLFALTLPIWAASKVNGWIFGTFLCKVVSLLKEVNFYSGILLLACISVDRYLAIVHACRTLTQKRHLVKFVCLGCWGLSMNLSLPFFLFRQAYHPNNSSPVCYEVLGNDTAKWRMVLRILPHTFGFIVPLFVMLFCYGFTLRTLFKAHGHYLSTQTSLSKDLNEKRDHMVLLEFVTAAGGGMGQKHRAMRVIFAVVLIFLLCWLPYNLVLLADTLMRTQVIQESCERRNNIGRALDATEILGFLHSCLNPIIYAFIGQNFRHGFLKILAMHGLVSKEFLARHRVTSYTSSSVNVSSNL

SEQ ID NO: 57 - protein, 396 aa, synthetic construct
MENETVSELNQTQLQPRAVVALEYQVVTILLVLIICGLGIVGNIMVVLVVMRTKHMRTPTNCYLVSLAVADLMVLVAAGLPNITDSIYGSWVYGYVGCLCITYLQYLGINASSCSITAFTIERYIAICHPIKAQFLCTFSRAKKIIIFVWAFTSLYCMLWFFLLDLNISTYKDAIVISCGYKISRNYYSPIYLMDFGVFYVVPMILATVLYGFIARILFLNPGHYLSTQTSLSKDLNEKRDHMVLLEFVTAAGGGVSSRKQVTKMLAVVVILFALLWMPYRTLVVVNSFLSSPFQENWFLLFCRICIYLNSAINPVIYNLMSQKFRAAFRKLCNCKQKPTEKPANYSVALNYSVIKESDHFSTELDDITVTDTYLSATKVSFDDTCLASEVSFSQS

SEQ ID NO: 58 - protein, 406 aa, synthetic construct
MRMEDEDYNTSISYGDEYPDYLDSIVVLEDLSPLEARVTRIFLVVVYSIVCFLGILGNGLVIIIATFKMKKTVNMVWFLNLAVADFLFNVFLPIHITYAAMDYHWVFGTAMCKISNFLLIHNMFTSVFLLTIISSDRCISVLLPVWSQNHRSVRLAYMACMVIWVLAFFLSSPSLVFRDTANLHGKISCFNNFSLSTPGSSSWPTHSQMDPVGYSRHMVVTVTRFLCGFLVPVLIITACYLTIVCKLQRNRGHYLSTQTSLSKDLNEKRDHMVLLEFVTAAGGGLAKTKKPFKIIVTIIITFFLCWCPYHTLNLLELHHTAMPGSVFSLGLPLATALAIANSCMNPILYVFMGQDFKKFKVALFSRLVNALSEDTGHSSYPSHRSFTKMSSMNERTSMNERETGML

SEQ ID NO: 59 - protein, 445 aa, synthetic construct
MQALNITPEQFSRLLRDHNLTREQFIALYRLRPLVYTPELPGRAKLALVLTGVLIFALALFGNALVFYVVTRSKAMRTVTNIFICSLALSDLLITFFCIPVTMLQNISDNWLGGAFICKMVPFVQSTAVVTEILTMTCIAVERHQGLVHPCKMKWQYTNRRAFTMLGVVWLVAVIVGSPMWHVQQLEIKYDFLYEKEHICCLEEWTSPVHQKIYTTFILVILFLLPLMVMLILYSKIGYELWIKKGHYLSTQTSLSKDLNEKRDHMVLLEFVTAAGGGARKKKRAVIMMVTVVALFAVCWAPFHVVHMMIEYSNFEKEYDDVTIKMIFAIVQIIGFSNSICNPIVYAFMNENFKKNVLSAVCYCIVNKTFSPAQRHGNSGITMMRKKAKFSLRENPVEETKGEAFSDGNIEVKLCEQTEEKKKLKRHLALFRSELAENSPLDSGH

SEQ ID NO: 60 - protein, 394 aa, synthetic construct
MDMADEPLNGSHTWLSIPFDLNGSVVSTNTSNQTEPYYDLTSNAVLTFIYFVVCIIGLCGNTLVIYVILRYAKMKTITNIYILNLAIADELFMLGLPFLAMQVALVHWPFGKAICRVVMTVDGINQFTSIFCLTVMSIDRYLAVVHPCKSAKWRRPRTAKMITMAVWGVSLLVILPIMIYAGLRSNQWGRSSCTINWPGESGAWYTGFIIYTFILGFLVPLTIICLCYLFIIIKVKSSGGHYLSTQTSLSKDLNEKRDHMVLLEFVTAAGGGKKSEKKVTRMVSIVVAVFIFCWLPFYIFNVSSVSMAISPTPALKGMFDFVVVLTYANSCANPILYAFLSDNFKKSFQNVLCLVKVSGTDDGERSDSKQDKSRLNETTETQRTLLNGDLQTSI

SEQ ID NO: 61 - protein, 331 aa, synthetic construct
MDLPPQLSFGLYVAAFALGFPLNVLAIRGATAHARLRLTPSLVYALNLGCSDLLLTVSLPLKAVEALASGAWPLPASLCPVFAVAHFFPLYAGGGFLAALSAGRYLGAAFPCGYQAFRRPCYSWGVCAAIWALVLCHLGLVFGLEAPGGWLDHSNTSLGINTPVNGSPVCLEAWDPASAGPARFSLSLLLFFLPLAITAFCYVGCLRALARSGGHYLSTQTSLSKDLNEKRDHMVLLEFVTAAGGGHRRKLRAAWVAGGALLTLLLCVGPYNASNVASFLYPNLGGSWRKLGLITGAWSVVLNPLVTGYLGRGPGLKTVCAARTQGGKSQK

SEQ ID NO: 62 - protein, 369 aa, synthetic construct
MEPHDSSHMDSEFRYTLFPIVYSIIFVLGVIANGYVLWVFARLYPCKKFNEIKIFMVNLTMADMLFLITLPLWIVYYQNQGNWILPKFLCNVAGCLFFINTYCSVAFLGVITYNRFQAVTRPCKTAQANTRKRGISLSLVIWVAIVGAASYFLILDSTNTVPDSAGSGNVTRCFEHYEKGSVPVLIIHIFIVFSFFLVFLIILFCNLVIIRTLLMQPGHYLSTQTSLSKDLNEKRDHMVLLEFVTAAGGGAEVKRRALWMVCTVLAVFIICFVPHHVVQLPWTLAELGFQDSKFHQAINDAHQVTLCLLSTNCVLDPVIYCFLTKKFRKHLTEKFYSMRSSRKCSRATTDTVTEVVVPFNQIPGNSLKN

SEQ ID NO: 63 - protein, 403 aa, synthetic construct
MTEVLWPAVPNGTDAAFLAGPGSSWGNSTVASTAAVSSSFKCALTKTGFQFYYLPAVYILVFIIGFLGNSVAIWMFVFHMKPWSGISVYMFNLALADFLYVLTLPALIFYYFNKTDWIFGDAMCKLQRFIFHVNLYGSILFLTCISAHRYSGVVYPCKSLGRLKKKNAICISVLVWLIVVVAISPILFYSGTGVRKNKTITCYDTTSDEYLRSYFIYSMCTTVAMFCVPLVLILGCYGLIVRALIYKDGHYLSTQTSLSKDLNEKRDHMVLLEFVTAAGGGSPLRRKSIYLVIIVLTVFAVSYIPFHVMKTMNLRARLDFQTPAMCAFNDRVYATYQVTRGLASLNSCVDPILYFLAGDTFRRRLSRATRKASRRSEANLQSKSEDMTLNILPEFKQNGDTSL

SEQ ID NO: 64 - protein, 393 aa, synthetic construct
MNRHHLQDHFLEIDKKNCCVFRDDFIVKVLPPVLGLEFIFGLLGNGLALWIFCFHLKSWKSSRIFLFNLAVADFLLIICLPFLMDNYVRRWDWKFGDIPCRLMLFMLAMNRQGSIIFLTVVAVDRYFRVVHPCHALNKISNRTAAIISCLLWGITIGLTVHLLKKKMPIQNGGANLCSSFSICHTFQWHEAMFLLEFFLPLGIILFCSARIIWSLRQRQGHYLSTQTSLSKDLNEKRDHMVLLEFVTAAGGGHAKIKRAITFIMVVAIVFVICFLPSVVVRIRIFWLLHTSGTQNCEVYRSVDLAFFITLSFTYMNSMLDPVVYYFSSPSFPNFFSTLINRCLQRKMTGEPDNNRSTSVELTGDPNKTRGAPEALMANSGEPWSPSYLGPTSP

SEQ ID NO: 65 - protein, 362 aa, synthetic construct
MLGIMAWNATCKNWLAAEAALEKYYLSIFYGIEFVVGVLGNTIVVYGYIFSLKNWNSSNIYLFNLSVSDLAFLCTLPMLIRSYANGNWIYGDVLCISNRYVLHANLYTSILFLTFISIDRYLIIKYPCREHLLQKKEFAILISLAIWVLVTLELLPILPLINPVITDNGTTCNDFASSGDPNYNLIYSMCLTLLGFLIPLFVMCFFYYKIALFLKQRNGHYLSTQTSLSKDLNEKRDHMVLLEFVTAAGGGLQKEEKPLNLVIMAVVIFSVLFTPYHVMRNVRIASRLGSWKQYQCTQVVINSFYIVTRPLAFLNSVINPVFYFLLGDHFRDMLMNQLRHNFKSLTSFSRWAHELLLSFREK

SEQ ID NO: 66 - protein, 357 aa, synthetic construct
EEGGDFDNYYGADNQSECEYTDWKSSGALIPAIYMLVFLLGTTGNGLVLWTVFRSSREKRRSADIFIASLAVADLTFVVTLPLWATYTYRDYDWPFGTFFCKLSSYLIFVNMYASVFCLTGLSFDRYLAIVRPVANARLRLRVSGAVATAVLWVLAALLAMPVMVLRTTGDLENTTKVQCYMDYSMVATVSSEWAWEVGLGVSSTTVGFVVPFTIMLTCYFFIAQTIAGHSGGHYLSTQTSLSKDLNEKRDHMVLLEFVTAAGGGGLRKRRRLLSIIVVLVVTFALCWMPYHLVKTLYMLGSLLHWPCDFDLFLMNIFPYCTCISYVNSCLNPFLYAFFDPRFRQACTSMLCCGQSR

SEQ ID NO: 67 - protein, 463 aa, synthetic construct
MASPSLPGSDCSQIIDHSHVPEFEVATWIKITLILVYLIIFVMGLLGNSATIRVTQVLQKKGYLQKEVTDHMVSLACSDILVFLIGMPMEFYSIIWNPLTTSSYTLSCKLHTFLFEACSYATLLHVLTLSFERYIAICHPCRYKAVSGPCQVKLLIGFVWVTSALVALPLLFAMGTEYPLVNVPSHRGLTCNRSSTRHHEQPETSNMSICTNLSSRWTVFQSSIFGAFVVYLVVLLSVAFMCWNMMQVLRRQLGHYLSTQTSLSKDLNEKRDHMVLLEFVTAAGLQKERQTIIFLRLIVVTLAVCWMPNQIRRIMAAAKPKHDWTRSYFRAYMILLPFSETFFYLSSVINPLLYTVSSQQFRRVFVQVLCCRLSLQHANHEKRLRVHAHSTTDSARFVQRPLLFASRRQSSARRTEKIFLSTFQSEAEPQSKSQSLSLESLEPNSGAKPANSAAENGFQEHEV

SEQ ID NO: 68 - protein, 347 aa, synthetic construct
MNSTGHLQDAPNATSLHVPHSQEGNSTSLQEGLQDLIHTATLVTCTFLLAVIFCLGSYGNFIVFLSFFDPAFRKFRTNFDFMILNLSFCDLFICGVTAPMFTFVLFFSSASSIPDAFCFTFHLTSSGFIIMSLKTVAVIALHRLRMVLGKCPNRTASFPCTVLLTLLLWATSFTLATLATLKTSKSHLCLPMSSLIAGKGKAILSLYVVDFTFCVAVVSVSYIMIAQTLRKNAGHYLSTQTSLSKDLNEKRDHMVLLEFVTAAGTAKDSKAVVTCVIIVLSVLVCCLPLGISLVQVVLSSNGSFILYQFELFGFTLIFFKSGLNPFIYSRNSAGLRRKVLWCLQYIG

SEQ ID NO: 69 - protein, 348 aa, synthetic construct
STPGVNSSASLSPDRLNSPVTIPAVMFIFGVVGNLVAIVVLCKSRKEQKETTFYTLVCGLAVTDLLGTLLVSPVTIATYMKGQWPGGQPLCEYSTFILLFFSLSGLSIICAMSVERYLAINHACFYSHYVDKRLAGLTLFAVYASNVLFCALPNMGLGSSRLQYPDTWCFIDWTTNVTAHAAYSYMYAGFSSFLILATVLCNVLVCGALRRQLGHYLSTQTSLSKDLNEKRDHMVLLEFVTAAGLQKEIQMVILLIATSLVVLICSIPLVVRVFVNQLYQPSLEREVSKNPDLQAIRIASVNPILDPWIYILLRKTVLSKAIEKIKCLFCRIGGSRRERSGQHCSDSQ

SEQ ID NO: 70 - protein, 385 aa, synthetic construct
ETPNTTEDYDTTTEFDYGDATPCQKVNERAFGAQLLPPLYSLVFVIGLVGNILVVLVLVQYKRLKNMTSIYLLNLAISDLLFLFTLPFWIDYKLKDDWVFGDAMCKILSGFYYTGLYSEIFFIILLTIDRYLAIVHACFALRARTVTFGVITSIIIWALAILASMPGLYFSKTQWEFTHHTCSLHFPHESLREWKLFQALKLNLFGLVLPLLVMIICYTGIIKILRRQLGHYLSTQTSLSKDLNEKRDHMVLLEFVTAAGLQKESKAVRLIFVIMIIFFLFWTPYNLTILISVFQDFLFTHECEQSRHLDLAVQVTEVIAYTHCCVNPVIYAFVGERFRKYLRQLFHRRVAVHLVKWLPFLSVDRLERVSSTSPSTGEHELSAGF

SEQ ID NO: 71 - protein, 390 aa, synthetic construct
NPTDIADTTLDESIYSNYYLYESIPKPCTKEGIKAFGELFLPPLYSLVFVFGLLGNSVVVLVLFKYKRLRSMTDVYLLNLAISDLLFVFSLPFWGYYAADQWVFGLGLCKMISWMYLVGFYSGIFFVMLMSIDRYLAIVHACFSLRARTLTYGVITSLATWSVAVFASLPGFLFSTCYTERNHTYCKTKYSLNSTTWKVLSSLEINILGLVIPLGIMLFCYSMIIRTLRRQLGHYLSTQTSLSKDLNEKRDHMVLLEFVTAAGLQKENKAVKMIFAVVVLFLGFWTPYNIVLFLETLVELEVLQDCTFERYLDYAIQATETLAFVHCCLNPIIYFFLGEKFRKYILQLFKTCRGLFVLCQYCGLLQIYSADTPSSSYTQSTMDHDLHDAL

SEQ ID NO: 72 - protein, 294 aa, synthetic construct
DLGKKLLEAARAGQDDEVRILMANGADVNAADDVGVTPLHLAAQRGHLEIVEVLLKYGADVNAADLWGQTPLHLAATAGHLEIVEVLLKNGADVNARDNIGHTPLHLAAWAGHLEIVEVLLKYGADVNAQDKFGKTPFDLAIDNGNEDIAEVLQKAAGGGSGGGDVNAYDEVGWTPLHKAAWGHLEKVEDLLKNGADVNAADIDGYTPLHLAAFSGHLEIVEVLLKYGADVNADDQAGFTPLHLAAIFGHLEIVEVLLKNGADVNAQDKFGKTPFDLAIDNGNEDIAEVLQKAA

SEQ ID NO: 73 - protein, 294 aa, synthetic construct
DLGKKLLEAARAGQDDEVRILMANGADVNAADDVGVTPLHLAAQRGHLEIVEVLLKYGADVNAADLWGQTPLHLAATAGHLEIVEVLLKNGADVNARDNIGHTPLHLAAWAGHLEIVEVLLKYGADVNAQDKFGKTPFDLAIDNGNEDIAEVLQKAAGGGSGGGDVNAYDEVGWTPLHKAAWGHLCKVEDLLKNGADVNAADIDGYTPLHLAAFSGHLEIVEVLLKYGADVNADDQAGFTPLHLAAIFGHLEIVEVLLKNGADVNAQDKFGKTPFDLAIDNGNEDIAEVLQKAA

SEQ ID NO: 74 - protein, 321 aa, synthetic construct
DLGKKLLEAARAGQDDEVRILMANGADVNAADDVGVTPLHLAAQRGHLEIVEVLLKYGADVNAADLWGQTPLHLAATAGHLEIVEVLLKNGADVNARDNIGHTPLHLAAWAGHLEIVEVLLKYGADVNAQDKFGKTPFDLAIDNGNEDIAEVLQKAAGGGSGGGDVNAYDEVGWTPLHKAAWGHLEKVEDLLKNGADVNAADIDGYTPLHLAAFSGHLEIVEVLLKYGADVNADDQAGFTPLHLAAIFGHLEIVEVLLKNGADVNAQDKFGKTPFDLAIDNGNEDIAEVLQKAASHHHHHHHHSGGGLNDIFEAQKIEWHE

SEQ ID NO: 75 - protein, 354 aa, synthetic construct
DYTLDLSVTTVTDYYYPDIFSSPCDAELIQTNGKLLLAVFYCLLFVFSLLGNSLVILVLVVCKKLRSITDVYLLNLALSDLLFVFSFPFQTYYLLDQWVFGTVMCKVVSGFYYIGFYSSMFFITLMSVDRYLAVVHAVYALKVRTIRMGTTLCLAVWLTAIMATIPLLVFYQVASEDGVLQCYSFYNQQTLKWKIFTNFKMNILGLLIPFTIFMFCYIKILHQLKRCQNHNKTKAIRLVLIVVIASLLFWVPFNVVLFLTSLHSMHILDGCSISQQLTYATHVTEIISFTHCCVNPVIYAFVGEKFKKHLSEIFQKSCSQIFNYLGRQMPRESCEKSSSCQQHSSRSSSVDYIL

SEQ ID NO: 76 - protein, 516 aa, synthetic construct
DYTLDLSVTTVTDYYYPDIFSSPCDAELIQTNGKLLLAVFYCLLFVFSLLGNSLVILVLVVCKKLRSITDVYLLNLALSDLLFVFSFPFQTYYLLDQWVFGTVMCKVVSGFYYIGFYSSMFFITLMSVDRYLAVVHAVYALKVRTIRMGTTLCLAVWLTAIMATIPLLVFYQVASEDGVLQCYSFYNQQTLKWKIFTNFKMNILGLLIPFTIFMFCYIKILHQLKRCQGNIFEMLRIDEGLRLKIYKDTEGYYTIGIGHLLTKSPSLNAAKSELDKAIGRNTNGVITKDEAEKLFNQDVDAAVRGILRNAKLKPVYDSLDAVRRAALINMVFQMGETGVAGFTNSLRMLQQKRWDEAAVNLAKSRWYNQTPNRAKRVITTFRTGTWDAYGNHNKTKAIRLVLIVVIASLLFWVPFNVVLFLTSLHSMHILDGCSISQQLTYATHVTEIISFTHCCVNPVIYAFVGEKFKKHLSEIFQKSCSQIFNYLGRQMPRESCEKSSSCQQHSSRSSSVDYIL

SEQ ID NO: 77 - protein, 410 aa, synthetic construct
DYTLDLSVTTVTDYYYPDIFSSPCDAELIQTNGKLLLAVFYCLLFVFSLLGNSLVILVLVVCKKLRSITDVYLLNLALSDLLFVFSFPFQTYYLLDQWVFGTVMCKVVSGFYYIGFYSSMFFITLMSVDRYLAVVHAVYALKVRTIRMGTTLCLAVWLTAIMATIPLLVFYQVASEDGVLQCYSFYNQQTLKWKIFTNFKMNILGLLIPFTIFMFCYIKILHQLKRCQGMKKYTCTVCGYIYNPEDGDPDNGVNPGTDFKDIPDDWVCPLCGVGKDQFEEVEEGNHNKTKAIRLVLIVVIASLLFWVPFNVVLFLTSLHSMHILDGCSISQQLTYATHVTEIISFTHCCVNPVIYAFVGEKFKKHLSEIFQKSCSQIFNYLGRQMPRESCEKSSSCQQHSSRSSSVDYIL

SEQ ID NO: 78 - protein, 462 aa, synthetic construct
DYTLDLSVTTVTDYYYPDIFSSPCDAELIQTNGKLLLAVFYCLLFVFSLLGNSLVILVLVVCKKLRSITDVYLLNLALSDLLFVFSFPFQTYYLLDQWVFGTVMCKVVSGFYYIGFYSSMFFITLMSVDRYLAVVHAVYALKVRTIRMGTTLCLAVWLTAIMATIPLLVFYQVASEDGVLQCYSFYNQQTLKWKIFTNFKMNILGLLIPFTIFMFCYIKILHQLKRCQGADLEDNWETLNDNLKVIEKADNAAQVKDALTKMRAAALDAQKATPPKLEDKSPDSPEMKDFRHGFDILVGQIDDALKLANEGKVKEAQAAAEQLKTTRNAYIQKYLGNHNKTKAIRLVLIVVIASLLFWVPFNVVLFLTSLHSMHILDGCSISQQLTYATHVTEIISFTHCCVNPVIYAFVGEKFKKHLSEIFQKSCSQIFNYLGRQMPRESCEKSSSCQQHSSRSSSVDYIL

SEQ ID NO: 79 - protein, 503 aa, synthetic construct
DYTLDLSVTTVTDYYYPDIFSSPCDAELIQTNGKLLLAVFYCLLFVFSLLGNSLVILVLVVCKKLRSITDVYLLNLALSDLLFVFSFPFQTYYLLDQWVFGTVMCKVVSGFYYIGFYSSMFFITLMSVDRYLAVVHAVYALKVRTIRMGTTLCLAVWLTAIMATIPLLVFYQVASEDGVLQCYSFYNQQTLKWKIFTNFKMNILGLLIPFTIFMFCYIKILHQLKRCQGAKALIVYGSTTGNTEYTAETIARELADAGYEVDSRDAASVEAGGLFEGFDLVLLGCSTWGDDSIELQDDFIPLFDSLEETGAQGRKVACFGCGDSSWEYFCGAVDAIEEKLKNLGAEIVQDGLRIDGDPRAARDDIVGWAHDVRGAIGNHNKTKAIRLVLIVVIASLLFWVPFNVVLFLTSLHSMHILDGCSISQQLTYATHVTEIISFTHCCVNPVIYAFVGEKFKKHLSEIFQKSCSQIFNYLGRQMPRESCEKSSSCQQHSSRSSSVDYIL

SEQ ID NO: 80 - protein, 552 aa, synthetic construct
DYTLDLSVTTVTDYYYPDIFSSPCDAELIQTNGKLLLAVFYCLLFVFSLLGNSLVILVLVVCKKLRSITDVYLLNLALSDLLFVFSFPFQTYYLLDQWVFGTVMCKVVSGFYYIGFYSSMFFITLMSVDRYLAVVHAVYALKVRTIRMGTTLCLAVWLTAIMATIPLLVFYQVASEDGVLQCYSFYNQQTLKWKIFTNFKMNILGLLIPFTIFMFCYIKILHQLKRCQGGIDCSFWNESYLTGSRDERKKSLLSKFGMDEGVTFMFIGRFDRGQKGVDVLLKAIEILSSKKEFQEMRFIIIGKGDPELEGWARSLEEKHGNVKVITEMLSREFVRELYGSVDFVIIPSYFEPFGLVALEAMCLGAIPIASAVGGLRDIITNETGILVKAGDPGELANAILKALELSRSDLSKFRENCKKRAMSFSGNHNKTKAIRLVLIVVIASLLFWVPFNVVLFLTSLHSMHILDGCSISQQLTYATHVTEIISFTHCCVNPVIYAFVGEKFKKHLSEIFQKSCSQIFNYLGRQMPRESCEKSSSCQQHSSRSSSVDYIL

SEQ ID NO: 81 - protein, 241 aa, synthetic construct
MVSKGEELFTGVVPILVELDGDVNGHKFSVSGEGEGDATYGKLTLKFICTTGKLPVPWPTLVTTLTYGVQCFSRYPDHMKQHDFFKSAMPEGYVQERTIFFKDDGNYKTRAEVKFEGDTLVNRIELKGIDFKEDGNILGHKLEYNYNSHNVYIMADKQKNGIKVNFKIRHNIEDGSVQLADHYQQNTPIGDGPVLLPDNHYLSTQSALSKDPNEKRDHMVLLEFVTAAGITLGMDELYKQA

SEQ ID NO: 82 - protein, 321 aa, synthetic construct
DLGKKLLEAARAGQDDEVRILMANGADVNAADDVGVTPLHLAAQRGHLEIVEVLLKYGADVNAADLWGQTPLHLAATAGHLEIVEVLLKNGADVNARDNIGHTPLHLAAWAGHLEIVEVLLKYGADVNAQDKFGKTPFDLAIDNGNEDIAEVLQKAAGGGSGGGDVNAYDEVGWTPLHKAAWGHLCKVEDLLKNGADVNAADIDGYTPLHLAAFSGHLEIVEVLLKYGADVNADDQAGFTPLHLAAIFGHLEIVEVLLKNGADVNAQDKFGKTPFDLAIDNGNEDIAEVLQKAASHHHHHHHHSGGGLNDIFEAQKIEWHE